European Patent Specification EP 3 313 988 B1, published March 6, 2024. Title: PRODUCTION OF NOSCAPINE. Applicant: Sun Pharmaceutical Industries Australia PTY Limited THE UNIVERSITY OF YORK. The sequence listing filed with the application follows.

SEQUENCE LISTING (42 sequences)

SEQ ID NO: 1 - DNA, 1737 bp, Papaver somniferum
atggagctccaatatatttcttattttcaaccaacttcctccgttgttgctcttctacttgctcttgtatccatcttatccagtgtcgttgttttgaggaagacatttttgaataactactcatcatcacctgcatcatccacaaaaacagcggtactttctcatcagcggcagcagtcgtgtgcattgccaatttccggtctcctccatattttcatgaataaaaacggcttaattcatgtaactcttggaaatatggctgataaatacggtccgattttcagtttcccaacaggtagccatagaactctcgttgtgagcagttgggagatggtaaaagagtgttttactggcaacaatgacactgctttctcaaaccgtcctatcccgttagcttttaagactatattttatgcatgcggtggcatagactcatacggtctttcgagtgtaccttatggaaaatattggagggagcttcgaaaggtctgtgtgcataacctcctgtctaatcaacaactactcaagttcagacacttgataatttctcaagtcgatacgtctttcaataagctgtatgagttatgcaaaaactctgaagacaaccagggaaactatactactactactaccgcagctggcatggtgagaatcgatgattggctcgccgaattatcgttcaatgtgataggaagaatagtctgcggattccaatcaggccctaagacaggtgctccaagcagggtggaacaatttaaagaagcaattaatgaagcatcttattttatgtcgacatctccagtgtcagataatgttccaatgctagggtggattgaccaattgacaggtcttacgagaaatatgaagcactgcggaaagaaattagacttggtggtcgagagcataattaatgatcatcgtcaaaagagacgattctctagaactaaaggaggagatgagaaggacgatgaacaagatgacttcatcgacatttgtttgtcaataatggagcaaccacagcttcctggcaacaataatccttctcagatacctatcaaatctattgtcctggacatgataggtgggggcactgacaccacaaaactgaccaccatctggaccctttccttgctgctgaacaacccccatgtgttggacaaggcaaaacaagaagtggatgcacactttcgaaccaaaaggagatcaacaaatgatgcagcagcagccgtggtggattttgatgatattcgtaaccttgtctacatccaggcaatcatcaaagaatcaatgcggttgtatccagccagccccgtggtggagcgactgagcggcgaagattgtgtggtcggtgggtttcatgtaccagcagggacgagattatgggctaacgtatggaagatgcaacgagaccctaaagtatgggatgatccattggtgtttcgaccagacagatttttgagcgatgaacagaagatggttgatgtaaggggtcaaaattatgagctgttaccatttggagccggtcgacgtgtatgtccaggtgtatccttctctttggatctaatgcaactggtactgactcgtcttattctcgagtttgaaatgaagtctcctagcgggaaagtggacatgacagcaacaccaggattaatgagttacaaggtgatcccccttgacattctgctcacccatcgtcgcataaagccgtgtgtgcagtcagcagcctctgagagagac

SEQ ID NO: 2 - DNA, 1740 bp, Papaver somniferum
atggagctccaatatatttcttattttcaaccaacttcctccgttgttgctcttctacttgctcttgtatccatcttatccagtgtcgttgttttgaggaagacatttttgaataactactcatcatcacctgcatcatccacaaaaacagcggtactttctcatcagcggcagcagtcgtgtgcattgccaatttccggtctcctccatattttcatgaataaaaacggcttaattcatgtaactcttggaaatatggctgataaatacggtccgattttcagtttcccaacaggtagccatagaactctcgttgtgagcagttgggagatggtaaaagagtgttttactggcaacaatgacactgctttctcaaaccgtcctatcccgttagcttttaagactatattctatgcatgcggtggcatagactcatacggtctttcgagtgtaccttatggaaaatattggagggagcttcgaaaggtctgtgtgcataacctcctgtctaatcaacaactactcaagttcagacacttgataatttctcaagtcgatacgtctttcaataagctgtatgagttatgcaaaaactctgaagacaaccatggaaactatactactactactactaccgcagctggcatggtgagaatcgatgattggctcgccgaattatcgttcaatgtgataggaagaatagtctgcggattccaatcaggccctaagacaggtgctccaagcagggtggaacaatttaaagaagcaattaatgaagcatcttattttatgtcgacatctccagtgtcagataatgttccaatgctagggtggattgaccaattgacaggtcttacgagaaatatgaagcactgcggaaagaaattagacttggtggtcgagagcataattaatgatcatcgtcaaaagagacgattctctagaactaaaggaggagatgagaaggacgatgaacaagatgacttcatcgacatttgtttgtcaataatggagcaaccacagcttcctggcaacaataatccttctcagatacctatcaaatctattgtcctggacatgataggtgggggcactgacaccacaaaactgaccaccatctggaccctttccttgctgctgaacaacccccatgtgttggacaaggcaaaacaagaagtggatgcacactttcgaaccaaaaggagatcaacaaatgatgcagcagcagccgtggtggattttgatgatattcgtaaccttgtctacatccaggcaatcatcaaagaatcaatgcggttgtatccagccagccccgtggtggagcgactgagcggcgaagattgtgtggtcggtgggtttcatgtaccagcagggacgagattatgggctaacgtatggaagatgcaacgagaccctaaagtatgggatgatccattggtgtttcgaccagacagatttttgagcgatgaacagaagatggttgatgtaaggggtcaaaattatgagctgttaccatttggagccggtcgacgtgtatgtccaggtgtatccttctctttggatctaatgcaactggtactgactcgtcttattctcgagtttgaaatgaagtctcctagcgggaaagtggacatgacagcaacaccaggattaatgagttacaaggtgatcccccttgacattctgctcacccatcgtcgcataaagccgtgtgtgcagtcagcagcctctgagagagac

SEQ ID NO: 3 - DNA, 1737 bp, Papaver somniferum
atggagctccaatatatttcttattttcaaccaacttcctccgttgttgctcttctacttgctcttgtatccatcttatccagtgtcgttgttttgaggaagacatttttgaataactactcatcatcacctgcatcatccacaaaaacagcggtactttctcatcagcggcagcagtcgtgtgcattgccaatttccggtctcctccatattttcatgaataaaaacggcttaattcatgtaactcttggaaatatggctgataaatacggtccgattttcagtttcccaacaggtagccatagaactctcgttgtgagcagttgggagatggtaaaagagtgttttactggcaacaatgacactgctttctcaaaccgtcctatcccgttagcttttaagactatattctatgcatgcggtggcatagactcatacggtctttcgagtgtaccttatggaaaatattggagggagcttcgaaaggtctgtgtgcataacctcctgtctaatcaacaactactcaagttcagacacttgataatttctcaagtcgatacgtctttcaataagctgtatgagttatgcaaaaactctgaagacaaccagggaaactatcctactactactaccgcagctggcatggtgagaatcgatgattggctcgccgaattatcgttcaatgtgataggaagaatagtctgcggattccaatcaggccctaagacaggtgctccaagcagggtggaacaatttaaagaagcaattaatgaagcatcttattttatgtcgacatctccagtgtcagataatgttccaatgctagggtggattgaccaattgacaggtcttacgagaaatatgaagcactgcggaaagaaattagacttggtggtcgagagcataattaatgatcatcgtcaaaagagacgattctctagaactaaaggaggagatgagaaggacgatgaacaagatgacttcatcgacatttgtttgtcaataatggagcaaccacagcttcctggcaacaataatccttctcagatacctatcaaatctattgtcctggacatgataggtgggggcactgacaccacaaaactgaccaccatctggaccctttccttgctgctgaacaacccccatgtgttggacaaggcaaaacaagaagtggatgcacactttcgaaccaaaaggagatcaacaaatgatgcagcagcagccgtggtggattttgatgatattcgtaaccttgtctacatccaggcaatcatcaaagaatcaatgcggttgtatccagccagccccgtggtggagcgactgagcggcgaagattgtgtggtcggtgggtttcatgtaccagcagggacgagattatgggctaacgtatggaagatgcaacgagaccctaaagtatgggatgatccattggtgtttcgaccagacagatttttgagcgatgaacagaagatggttgatgtaaggggtcaaaattatgagctgttaccatttggagccggtcgacgtgtatgtccaggtgtatccttctctttggatctaatgcaactggtactgactcgtcttattctcgagtttgaaatgaagtctcctagcgggaaagtggacatgacagcaacaccaggattaatgagttacaaggtgatcccccttgacattctgctcacccatcgtcgcataaagccgtgtgtgcagtcagcagcctctgagagagac

SEQ ID NO: 4 - DNA, 966 bp, Papaver somniferum
atggagagtagtggtgtaccagtaatcactctgggctcgggcaaggtgatgcctgttcttggcatgggaacatttgagaaagttggtaaagggtccgaaagagagaggttggcgattttaaaagcgatagaggtgggttacagatacttcgatacagctgctgcatacgaaactgaagaggttcttggagaagctattgctgaagcacttcaacttggcctagtcaaatctcgagatgaacttttcatcagttccatgctctggtgcactgatgctcacgctgatcgtgtcctcctcgctcttcagaattcgctgaggaatcttaaattggagtatgtggatctatatatgttacccttcccggcaagcttgaagcctgggaagataacgatggacataccagaggaagatatttgtcgcatggactacaggtctgtatgggcagccatggaagagtgtcaaaaccttggcttcactaaatcaatcggtgttagcaatttctcctgcaaaaagcttcaggaattgatggcgactgccaacatccctccagctgtgaatcaagtggagatgagcccggctttccaacaaaagaagctgagagagtattgcaacgcaaataatatattagtcagtgcaatctctgtactgggatcaaacggaaccccatggggctccaatgcagttttgggttctgaggtgcttaagaaaattgctatggccaaaggaaaatctgttgctcaggttagtatgagatgggtttacgagcaaggcgcgagtcttgtggtaaaaagtttcagtgaagagagattgagggaaaacttgaacatatttgactgggaactcactaaggaagaccatgaaaagatcggtgagattccacagtgcagaatcttgagtgcttattttttggtctcacctaatggacctttcaaatctcaagaagagttgtgggatgatgaagcttga

SEQ ID NO: 5 - DNA, 966 bp, Papaver somniferum
atggagagtagtggtgtaccagtaattactctgagctcgggcaagttgatgcctgttctgggcatgggaacatttgagaaagttggtaaagggtccgaaagagagaggttggtgattttaaaagcgatagaggtgggttacagatacttcgatacagctgctgcatacgaaactgaagaggttcttggagaagctattgctgaagcactccaacttggcctaatcaaatctcgagatgaacttttcatcagttccatgctctggtgcactgatgctcatcctgatcgtgtcctcctcgctcttcagaattctctgaggaatcttaaattggagtatctggatctatatatgttacccttcccggtaagcttgaagccagggaagataacgatggacatacaagaggaagatatttgtcgcatggactacaggtctgtatgggcagccatggaagagtgtcagaaccttggcttcactaaatcaatcggtgttagtaatttctcctgcaaaaagcttcaggaattgatggcgaccgccaacatccctccagatgtgaatcaagtggagatgagcccggctttccaacaaaagaagctgagagattattgcaacgcaaataatatactagtcagtgcagtctctatactgggatcaaacggaaccccatggggctccaatgcagttttgggttctgaggtgcttaggaaaattgctatggccaaaggaaaatctgttgctcaggttagtatgagatgggtttacgatcaaggcgcgagtcttgtggtaaaaagtttcagtgaagagagattgagggaaaacttgaacatatttgactgggaactcactaaggaagaccatgaaaagatcggtgagattccacagtgcagaatcttgagtgcttattttttggtctcacctaatggacctttcaaatctcaagaagagttgtgggatgacgaagcttga

SEQ ID NO: 6 - DNA, 2703 bp, Papaver somniferum
atggagctccaatatatttcttattttcaaccaacttcctccgttgttgctcttctacttgctcttgtatccatcttatccagtgtcgttgttttgaggaagacatttttgaataactactcatcatcacctgcatcatccacaaaaacagcggtactttctcatcagcggcagcagtcgtgtgcattgccaatttccggtctcctccatattttcatgaataaaaacggcttaattcatgtaactcttggaaatatggctgataaatacggtccgattttcagtttcccaacaggtagccatagaactctcgttgtgagcagttgggagatggtaaaagagtgttttactggcaacaatgacactgctttctcaaaccgtcctatcccgttagcttttaagactatattttatgcatgcggtggcatagactcatacggtctttcgagtgtaccttatggaaaatattggagggagcttcgaaaggtctgtgtgcataacctcctgtctaatcaacaactactcaagttcagacacttgataatttctcaagtcgatacgtctttcaataagctgtatgagttatgcaaaaactctgaagacaaccagggaaactatactactactactaccgcagctggcatggtgagaatcgatgattggctcgccgaattatcgttcaatgtgataggaagaatagtctgcggattccaatcaggccctaagacaggtgctccaagcagggtggaacaatttaaagaagcaattaatgaagcatcttattttatgtcgacatctccagtgtcagataatgttccaatgctagggtggattgaccaattgacaggtcttacgagaaatatgaagcactgcggaaagaaattagacttggtggtcgagagcataattaatgatcatcgtcaaaagagacgattctctagaactaaaggaggagatgagaaggacgatgaacaagatgacttcatcgacatttgtttgtcaataatggagcaaccacagcttcctggcaacaataatccttctcagatacctatcaaatctattgtcctggacatgataggtgggggcactgacaccacaaaactgaccaccatctggaccctttccttgctgctgaacaacccccatgtgttggacaaggcaaaacaagaagtggatgcacactttcgaaccaaaaggagatcaacaaatgatgcagcagcagccgtggtggattttgatgatattcgtaaccttgtctacatccaggcaatcatcaaagaatcaatgcggttgtatccagccagccccgtggtggagcgactgagcggcgaagattgtgtggtcggtgggtttcatgtaccagcagggacgagattatgggctaacgtatggaagatgcaacgagaccctaaagtatgggatgatccattggtgtttcgaccagacagatttttgagcgatgaacagaagatggttgatgtaaggggtcaaaattatgagctgttaccatttggagccggtcgacgtgtatgtccaggtgtatccttctctttggatctaatgcaactggtactgactcgtcttattctcgagtttgaaatgaagtctcctagcgggaaagtggacatgacagcaacaccaggattaatgagttacaaggtgatcccccttgacattctgctcacccatcgtcgcataaagccgtgtgtgcagtcagcagcctctgagagagacatggagagtagtggtgtaccagtaatcactctgggctcgggcaaggtgatgcctgttctgggcatgggaacatttgagaaagttggtaaagggtccgaaagagagaggttggcgattttaaaagcgatagaggtgggttacagatacttcgatacagctgctgcatacgaaactgaagaggttcttggagaagctattgctgaagcacttcaacttggcctagtcaaatctcgagatgaacttttcatcagttccatgctctggtgcactgatgctcacgctgatcgtgtcctcctcgctcttcagaattcgctgaggaatcttaaattggagtatgtggatctatatatgttacccttcccggcaagcttgaagcctgggaagataacgatggacataccagaggaagatatttgtcgcatggactacaggtctgtatgggcagccatggaagagtgtcaaaaccttggcttcactaaatcaatcggtgttagcaatttctcctgcaaaaagcttcaggaattgatggcgaccgccaacatccctccagctgtgaatcaagtggagatgagcccggctttccaacaaaagaagctgagagagtattgcaacgcaaataatatattagtcagtgcaatctctgtactgggatcaaacggaaccccatggggctccaatgcagttttgggttctgaggtgcttaagaaaattgctatggccaaaggaaaatctgttgctcaggttagtatgagatgggtttacgagcaaggcgcgagtcttgtggtaaaaagtttcagtgaagagagattgagggaaaacttgaacatatttgactgggaactcactaaggaagaccatgaaaagatcggtgagattccacagtgcagaatcttgagtgcttattttttggtctcacctaatggacctttcaaatctcaagaagagttgtgggatgatgaagcttga

SEQ ID NO: 7 - DNA, 2706 bp, Papaver somniferum
atggagctccaatatatttcttattttcaaccaacttcctccgttgttgctcttctacttgctcttgtatccatcttatccagtgtcgttgttttgaggaagacatttttgaataactactcatcatcacctgcatcatccacaaaaacagcggtactttctcatcagcggcagcagtcgtgtgcattgccaatttccggtctcctccatattttcatgaataaaaacggcttaattcatgtaactcttggaaatatggctgataaatacggtccgattttcagtttcccaacaggtagccatagaactctcgttgtgagcagttgggagatggtaaaagagtgttttactggcaacaatgacactgctttctcaaaccgtcctatcccgttagcttttaagactatattctatgcatgcggtggcatagactcatacggtctttcgagtgtaccttatggaaaatattggagggagcttcgaaaggtctgtgtgcataacctcctgtctaatcaacaactactcaagttcagacacttgataatttctcaagtcgatacgtctttcaataagctgtatgagttatgcaaaaactctgaagacaaccatggaaactatactactactactactaccgcagctggcatggtgagaatcgatgattggctcgccgaattatcgttcaatgtgataggaagaatagtctgcggattccaatcaggccctaagacaggtgctccaagcagggtggaacaatttaaagaagcaattaatgaagcatcttattttatgtcgacatctccagtgtcagataatgttccaatgctagggtggattgaccaattgacaggtcttacgagaaatatgaagcactgcggaaagaaattagacttggtggtcgagagcataattaatgatcatcgtcaaaagagacgattctctagaactaaaggaggagatgagaaggacgatgaacaagatgacttcatcgacatttgtttgtcaataatggagcaaccacagcttcctggcaacaataatccttctcagatacctatcaaatctattgtcctggacatgataggtgggggcactgacaccacaaaactgaccaccatctggaccctttccttgctgctgaacaacccccatgtgttggacaaggcaaaacaagaagtggatgcacactttcgaaccaaaaggagatcaacaaatgatgcagcagcagccgtggtggattttgatgatattcgtaaccttgtctacatccaggcaatcatcaaagaatcaatgcggttgtatccagccagccccgtggtggagcgactgagcggcgaagattgtgtggtcggtgggtttcatgtaccagcagggacgagattatgggctaacgtatggaagatgcaacgagaccctaaagtatgggatgatccattggtgtttcgaccagacagatttttgagcgatgaacagaagatggttgatgtaaggggtcaaaattatgagctgttaccatttggagccggtcgacgtgtatgtccaggtgtatccttctctttggatctaatgcaactggtactgactcgtcttattctcgagtttgaaatgaagtctcctagcgggaaagtggacatgacagcaacaccaggattaatgagttacaaggtgatcccccttgacattctgctcacccatcgtcgcataaagccgtgtgtgcagtcagcagcctctgagagagacatggagagtagtggtgtaccagtaatcactctgggctcgggcaaggtgatgcctgttcttggcatgggaacatttgagaaagttggtaaagggtccgaaagagagaggttggcgattttaaaagcgatagaggtgggttacagatacttcgatacagctgctgcatacgaaactgaagaggttcttggagaagctattgctgaagcacttcaacttggcctagtcaaatctcgagatgaacttttcatcagttccatgctctggtgcactgatgctcacgctgatcgtgtcctcctcgctcttcagaattcgctgaggaatcttaaattggagtatgtggatctatatatgttacccttcccggcaagcttgaagcctgggaagataacgatggacataccagaggaagatatttgtcgcatggactacaggtctgtatgggcagccatggaagagtgtcaaaaccttggcttcactaaatcaatcggtgttagcaatttctcctgcaaaaagcttcaggaattgatggcgactgccaacatccctccagctgtgaatcaagtggagatgagcccggctttccaacaaaagaagctgagagagtattgcaacgcaaataatatattagtcagtgcaatctctgtactgggatcaaacggaaccccatggggctccaatgcagttttgggttctgaggtgcttaagaaaattgctatggccaaaggaaaatctgttgctcaggttagtatgagatgggtttacgagcaaggcgcgagtcttgtggtaaaaagtttcagtgaagagagattgagggaaaacttgaacatatttgactgggaactcactaaggaagaccatgaaaagatcggtgagattccacagtgcagaatcttgagtgcttattttttggtctcacctaatggacctttcaaatctcaagaagagttgtgggatgatgaagcttga

SEQ ID NO: 8 - DNA, 2703 bp, Papaver somniferum
atggagctccaatatatttcttattttcaaccaacttcctccgttgttgctcttctacttgctcttgtatccatcttatccagtgtcgttgttttgaggaagacatttttgaataactactcatcatcacctgcatcatccacaaaaacagcggtactttctcatcagcggcagcagtcgtgtgcattgccaatttccggtctcctccatattttcatgaataaaaacggcttaattcatgtaactcttggaaatatggctgataaatacggtccgattttcagtttcccaacaggtagccatagaactctcgttgtgagcagttgggagatggtaaaagagtgttttactggcaacaatgacactgctttctcaaaccgtcctatcccgttagcttttaagactatattctatgcatgcggtggcatagactcatacggtctttcgagtgtaccttatggaaaatattggagggagcttcgaaaggtctgtgtgcataacctcctgtctaatcaacaactactcaagttcagacacttgataatttctcaagtcgatacgtctttcaataagctgtatgagttatgcaaaaactctgaagacaaccagggaaactatcctactactactaccgcagctggcatggtgagaatcgatgattggctcgccgaattatcgttcaatgtgataggaagaatagtctgcggattccaatcaggccctaagacaggtgctccaagcagggtggaacaatttaaagaagcaattaatgaagcatcttattttatgtcgacatctccagtgtcagataatgttccaatgctagggtggattgaccaattgacaggtcttacgagaaatatgaagcactgcggaaagaaattagacttggtggtcgagagcataattaatgatcatcgtcaaaagagacgattctctagaactaaaggaggagatgagaaggacgatgaacaagatgacttcatcgacatttgtttgtcaataatggagcaaccacagcttcctggcaacaataatccttctcagatacctatcaaatctattgtcctggacatgataggtgggggcactgacaccacaaaactgaccaccatctggaccctttccttgctgctgaacaacccccatgtgttggacaaggcaaaacaagaagtggatgcacactttcgaaccaaaaggagatcaacaaatgatgcagcagcagccgtggtggattttgatgatattcgtaaccttgtctacatccaggcaatcatcaaagaatcaatgcggttgtatccagccagccccgtggtggagcgactgagcggcgaagattgtgtggtcggtgggtttcatgtaccagcagggacgagattatgggctaacgtatggaagatgcaacgagaccctaaagtatgggatgatccattggtgtttcgaccagacagatttttgagcgatgaacagaagatggttgatgtaaggggtcaaaattatgagctgttaccatttggagccggtcgacgtgtatgtccaggtgtatccttctctttggatctaatgcaactggtactgactcgtcttattctcgagtttgaaatgaagtctcctagcgggaaagtggacatgacagcaacaccaggattaatgagttacaaggtgatcccccttgacattctgctcacccatcgtcgcataaagccgtgtgtgcagtcagcagcctctgagagagacatggagagtagtggtgtaccagtaatcactctgggctcgggcaaggtgatgcctgttctgggcatgggaacatttgagaaagttggtaaagggtccgaaagagagaggttggcgattttaaaagcgatagaggtgggttacagatacttcgatacagctgctgcatacgaaactgaagaggttcttggagaagctattgctgaagcacttcaacttggcctagtcaaatctcgagatgaacttttcatcagttccatgctctggtgcactgatgctcacgctgatcgtgtcctcctcgctcttcagaattcgctgaggaatcttaaattggagtatgtggatctatatatgttacccttcccggcaagcttgaagcctgggaagataacgatggacataccagaggaagatatttgtcgcatggactacaggtctgtatgggcagccatggaagagtgtcaaaaccttggcttcactaaatcaatcggtgttagcaatttctcctgcaaaaagcttcaggaattgatggcgaccgccaacatccctccagctgtgaatcaagtggagatgagcccggctttccaacaaaagaagctgagagagtattgcaacgcaaataatatattagtcagtgcaatctctgtactgggatcaaacggaaccccatggggctccaatgcagttttgggttctgaggtgcttaagaaaattgctatggccaaaggaaaatctgttgctcaggttagtatgagatgggtttacgagcaaggcgcgagtcttgtggtaaaaagtttcagtgaagagagattgagggaaaacttgaacatatttgactgggaactcactaaggaagaccatgaaaagatcggtgagattccacagtgcagaatcttgagtgcttattttttggtctcacctaatggacctttcaaatctcaagaagagttgtgggatgatgaagcttga

SEQ ID NO: 9 - protein, 900 aa, Papaver somniferum
MELQYISYFQPTSSVVALLLALVSILSSVVVLRKTFLNNYSSSPASSTKTAVLSHQRQQSCALPISGLLHIFMNKNGLIHVTLGNMADKYGPIFSFPTGSHRTLVVSSWEMVKECFTGNNDTAFSNRPIPLAFKTIFYACGGIDSYGLSSVPYGKYWRELRKVCVHNLLSNQQLLKFRHLIISQVDTSFNKLYELCKNSEDNQGNYTTTTTAAGMVRIDDWLAELSFNVIGRIVCGFQSGPKTGAPSRVEQFKEAINEASYFMSTSPVSDNVPMLGWIDQLTGLTRNMKHCGKKLDLVVESIINDHRQKRRFSRTKGGDEKDDEQDDFIDICLSIMEQPQLPGNNNPSQIPIKSIVLDMIGGGTDTTKLTTIWTLSLLLNNPHVLDKAKQEVDAHFRTKRRSTNDAAAAVVDFDDIRNLVYIQAIIKESMRLYPASPVVERLSGEDCVVGGFHVPAGTRLWANVWKMQRDPKVWDDPLVFRPDRFLSDEQKMVDVRGQNYELLPFGAGRRVCPGVSFSLDLMQLVLTRLILEFEMKSPSGKVDMTATPGLMSYKVIPLDILLTHRRIKPCVQSAASERDMESSGVPVITLGSGKVMPVLGMGTFEKVGKGSERERLAILKAIEVGYRYFDTAAAYETEEVLGEAIAEALQLGLVKSRDELFISSMLWCTDAHADRVLLALQNSLRNLKLEYVDLYMLPFPASLKPGKITMDIPEEDICRMDYRSVWAAMEECQNLGFTKSIGVSNFSCKKLQELMATANIPPAVNQVEMSPAFQQKKLREYCNANNILVSAISVLGSNGTPWGSNAVLGSEVLKKIAMAKGKSVAQVSMRWVYEQGASLVVKSFSEERLRENLNIFDWELTKEDHEKIGEIPQCRILSAYFLVSPNGPFKSQEELWDDEA

SEQ ID NO: 10 - protein, 901 aa, Papaver somniferum
MELQYISYFQPTSSVVALLLALVSILSSVVVLRKTFLNNYSSSPASSTKTAVLSHQRQQSCALPISGLLHIFMNKNGLIHVTLGNMADKYGPIFSFPTGSHRTLVVSSWEMVKECFTGNNDTAFSNRPIPLAFKTIFYACGGIDSYGLSSVPYGKYWRELRKVCVHNLLSNQQLLKFRHLIISQVDTSFNKLYELCKNSEDNHGNYTTTTTTAAGMVRIDDWLAELSFNVIGRIVCGFQSGPKTGAPSRVEQFKEAINEASYFMSTSPVSDNVPMLGWIDQLTGLTRNMKHCGKKLDLVVESIINDHRQKRRFSRTKGGDEKDDEQDDFIDICLSIMEQPQLPGNNNPSQIPIKSIVLDMIGGGTDTTKLTTIWTLSLLLNNPHVLDKAKQEVDAHFRTKRRSTNDAAAAVVDFDDIRNLVYIQAIIKESMRLYPASPVVERLSGEDCVVGGFHVPAGTRLWANVWKMQRDPKVWDDPLVFRPDRFLSDEQKMVDVRGQNYELLPFGAGRRVCPGVSFSLDLMQLVLTRLILEFEMKSPSGKVDMTATPGLMSYKVIPLDILLTHRRIKPCVQSAASERDMESSGVPVITLGSGKVMPVLGMGTFEKVGKGSERERLAILKAIEVGYRYFDTAAAYETEEVLGEAIAEALQLGLVKSRDELFISSMLWCTDAHADRVLLALQNSLRNLKLEYVDLYMLPFPASLKPGKITMDIPEEDICRMDYRSVWAAMEECQNLGFTKSIGVSNFSCKKLQELMATANIPPAVNQVEMSPAFQQKKLREYCNANNILVSAISVLGSNGTPWGSNAVLGSEVLKKIAMAKGKSVAQVSMRWVYEQGASLVVKSFSEERLRENLNIFDWELTKEDHEKIGEIPQCRILSAYFLVSPNGPFKSQEELWDDEA

SEQ ID NO: 11 - protein, 900 aa, Papaver somniferum
MELQYISYFQPTSSVVALLLALVSILSSVVVLRKTFLNNYSSSPASSTKTAVLSHQRQQSCALPISGLLHIFMNKNGLIHVTLGNMADKYGPIFSFPTGSHRTLVVSSWEMVKECFTGNNDTAFSNRPIPLAFKTIFYACGGIDSYGLSSVPYGKYWRELRKVCVHNLLSNQQLLKFRHLIISQVDTSFNKLYELCKNSEDNQGNYPTTTTAAGMVRIDDWLAELSFNVIGRIVCGFQSGPKTGAPSRVEQFKEAINEASYFMSTSPVSDNVPMLGWIDQLTGLTRNMKHCGKKLDLVVESIINDHRQKRRFSRTKGGDEKDDEQDDFIDICLSIMEQPQLPGNNNPSQIPIKSIVLDMIGGGTDTTKLTTIWTLSLLLNNPHVLDKAKQEVDAHFRTKRRSTNDAAAAVVDFDDIRNLVYIQAIIKESMRLYPASPVVERLSGEDCVVGGFHVPAGTRLWANVWKMQRDPKVWDDPLVFRPDRFLSDEQKMVDVRGQNYELLPFGAGRRVCPGVSFSLDLMQLVLTRLILEFEMKSPSGKVDMTATPGLMSYKVIPLDILLTHRRIKPCVQSAASERDMESSGVPVITLGSGKVMPVLGMGTFEKVGKGSERERLAILKAIEVGYRYFDTAAAYETEEVLGEAIAEALQLGLVKSRDELFISSMLWCTDAHADRVLLALQNSLRNLKLEYVDLYMLPFPASLKPGKITMDIPEEDICRMDYRSVWAAMEECQNLGFTKSIGVSNFSCKKLQELMATANIPPAVNQVEMSPAFQQKKLREYCNANNILVSAISVLGSNGTPWGSNAVLGSEVLKKIAMAKGKSVAQVSMRWVYEQGASLVVKSFSEERLRENLNIFDWELTKEDHEKIGEIPQCRILSAYFLVSPNGPFKSQEELWDDEA

SEQ ID NO: 12 - protein, 579 aa, Papaver somniferum
MELQYISYFQPTSSVVALLLALVSILSSVVVLRKTFLNNYSSSPASSTKTAVLSHQRQQSCALPISGLLHIFMNKNGLIHVTLGNMADKYGPIFSFPTGSHRTLVVSSWEMVKECFTGNNDTAFSNRPIPLAFKTIFYACGGIDSYGLSSVPYGKYWRELRKVCVHNLLSNQQLLKFRHLIISQVDTSFNKLYELCKNSEDNQGNYTTTTTAAGMVRIDDWLAELSFNVIGRIVCGFQSGPKTGAPSRVEQFKEAINEASYFMSTSPVSDNVPMLGWIDQLTGLTRNMKHCGKKLDLVVESIINDHRQKRRFSRTKGGDEKDDEQDDFIDICLSIMEQPQLPGNNNPSQIPIKSIVLDMIGGGTDTTKLTTIWTLSLLLNNPHVLDKAKQEVDAHFRTKRRSTNDAAAAVVDFDDIRNLVYIQAIIKESMRLYPASPVVERLSGEDCVVGGFHVPAGTRLWANVWKMQRDPKVWDDPLVFRPDRFLSDEQKMVDVRGQNYELLPFGAGRRVCPGVSFSLDLMQLVLTRLILEFEMKSPSGKVDMTATPGLMSYKVIPLDILLTHRRIKPCVQSAASERD

SEQ ID NO: 13 - protein, 580 aa, Papaver somniferum
MELQYISYFQPTSSVVALLLALVSILSSVVVLRKTFLNNYSSSPASSTKTAVLSHQRQQSCALPISGLLHIFMNKNGLIHVTLGNMADKYGPIFSFPTGSHRTLVVSSWEMVKECFTGNNDTAFSNRPIPLAFKTIFYACGGIDSYGLSSVPYGKYWRELRKVCVHNLLSNQQLLKFRHLIISQVDTSFNKLYELCKNSEDNHGNYTTTTTTAAGMVRIDDWLAELSFNVIGRIVCGFQSGPKTGAPSRVEQFKEAINEASYFMSTSPVSDNVPMLGWIDQLTGLTRNMKHCGKKLDLVVESIINDHRQKRRFSRTKGGDEKDDEQDDFIDICLSIMEQPQLPGNNNPSQIPIKSIVLDMIGGGTDTTKLTTIWTLSLLLNNPHVLDKAKQEVDAHFRTKRRSTNDAAAAVVDFDDIRNLVYIQAIIKESMRLYPASPVVERLSGEDCVVGGFHVPAGTRLWANVWKMQRDPKVWDDPLVFRPDRFLSDEQKMVDVRGQNYELLPFGAGRRVCPGVSFSLDLMQLVLTRLILEFEMKSPSGKVDMTATPGLMSYKVIPLDILLTHRRIKPCVQSAASERD

SEQ ID NO: 14 - protein, 579 aa, Papaver somniferum
MELQYISYFQPTSSVVALLLALVSILSSVVVLRKTFLNNYSSSPASSTKTAVLSHQRQQSCALPISGLLHIFMNKNGLIHVTLGNMADKYGPIFSFPTGSHRTLVVSSWEMVKECFTGNNDTAFSNRPIPLAFKTIFYACGGIDSYGLSSVPYGKYWRELRKVCVHNLLSNQQLLKFRHLIISQVDTSFNKLYELCKNSEDNQGNYPTTTTAAGMVRIDDWLAELSFNVIGRIVCGFQSGPKTGAPSRVEQFKEAINEASYFMSTSPVSDNVPMLGWIDQLTGLTRNMKHCGKKLDLVVESIINDHRQKRRFSRTKGGDEKDDEQDDFIDICLSIMEQPQLPGNNNPSQIPIKSIVLDMIGGGTDTTKLTTIWTLSLLLNNPHVLDKAKQEVDAHFRTKRRSTNDAAAAVVDFDDIRNLVYIQAIIKESMRLYPASPVVERLSGEDCVVGGFHVPAGTRLWANVWKMQRDPKVWDDPLVFRPDRFLSDEQKMVDVRGQNYELLPFGAGRRVCPGVSFSLDLMQLVLTRLILEFEMKSPSGKVDMTATPGLMSYKVIPLDILLTHRRIKPCVQSAASERD

SEQ ID NO: 15 - protein, 321 aa, Papaver somniferum
MESSGVPVITLGSGKVMPVLGMGTFEKVGKGSERERLAILKAIEVGYRYFDTAAAYETEEVLGEAIAEALQLGLVKSRDELFISSMLWCTDAHADRVLLALQNSLRNLKLEYVDLYMLPFPASLKPGKITMDIPEEDICRMDYRSVWAAMEECQNLGFTKSIGVSNFSCKKLQELMATANIPPAVNQVEMSPAFQQKKLREYCNANNILVSAISVLGSNGTPWGSNAVLGSEVLKKIAMAKGKSVAQVSMRWVYEQGASLVVKSFSEERLRENLNIFDWELTKEDHEKIGEIPQCRILSAYFLVSPNGPFKSQEELWDDEA

SEQ ID NO: 16 - protein, 321 aa, Papaver somniferum
MESSGVPVITLSSGKLMPVLGMGTFEKVGKGSERERLVILKAIEVGYRYFDTAAAYETEEVLGEAIAEALQLGLIKSRDELFISSMLWCTDAHPDRVLLALQNSLRNLKLEYLDLYMLPFPVSLKPGKITMDIQEEDICRMDYRSVWAAMEECQNLGFTKSIGVSNFSCKKLQELMATANIPPDVNQVEMSPAFQQKKLRDYCNANNILVSAVSILGSNGTPWGSNAVLGSEVLRKIAMAKGKSVAQVSMRWVYDQGASLVVKSFSEERLRENLNIFDWELTKEDHEKIGEIPQCRILSAYFLVSPNGPFKSQEELWDDEA

SEQ ID NO: 17 - DNA, 2306 bp, Papaver somniferum
cacaccaaacttgatcattgtcataaaaaacagtcctaattgtcatcaatcaaaaacagtcctaacatggctaccaatggcgaaattttcaatacctatggtcataatcatcaatcagccacagtcactaaaatcactgcttctaatgaaagcagcaatggtgtctgttatctttcagaaacggctaacttggggaagttaatatgcattccaatggcactaagagctgcgatggagctaaatgtgttccaacttatctcaaagttcggaactgacgcaaaagtttcggcttctgaaattgcctctaaaatgccaaacgcgaagaataatcctgaagcagctatgtatttggatagaattcttcgactgctcggggcaagttctattctttctgtttctactacaaaaaaatcaatcaacagaggaggagatgatgtagtagtacatgagaagctttatgggttaacaaattcgtcgtgttgtttggtccctcgacaagaagacggggtgtcattagtcgaagaattgctattcacatctgacaaggttgttgtggatagttttttcaaactgaaatgtgtggtggaagaaaaagacagtgtgccatttgaggttgctcatggtgctaaaatctttgagtatgctgctacagaaccaagaatgaatcaagtatttaacgatggaatggcagttttctctattgttgtttttgaggctgtttttagagtttacgatggatttcttgatatgaaagaattgttagatgttggtggtggtattggtacttcggttagtaagattgttgctaaataccctttgattcgcggtgtcaacttcgacttgcctcatgttatttctgttgcccctcaatacccaggtataccttcttcttcttttttctgaaaagaacgggttcgaatttttacagaattttttttctcattcgatactcaagcaactctattaaagtatactgtgtaataatgcatgcaggtgtagagcatgttgcaggagatatgttcgaggaagtcccaaagggtcaaaacatgttgctaaaagtaagctaaccatactcaattttcttaataattaggaaaattgcaaaaaccgtcacaatattataaaggcatctgaagtgccatcactcagataccgatgctatgtactctatacattgacaaaattccatggtatcaagtctcaacctgccggttataataatttttttcaggctttctttaaaagaaattattttgaatggtaaaaatcatcattatattggagaaaagtgcagatcttgctacattaaaatttataatataataaaacatttgtttatggttgtttgaaaaaaaaaatctcattgttaatgcatctttctaagttaatggtgattaatggtgaataatatgatatcttattaccgtcttgacacttttttttttgtcgtagacaaaatatttccaacttttctatattaataaaatcagaaatatttcatttatatgaatattaaaataagaaggtgcatgagtaatattccaaatttcttaaagcgttttttatagcagtacggcgttttctcaaatcttattaacccataattaaagggtttccgtaaattaaattgagggatatcaaaacaaaaacaaaaaatagggttattttgcagtaaaatcaataaccccttatcatatgaaaaggataacttagtctaccccaatttggagagatatgggcaattattgtattactagttcgtttgagcattgataatatttttcattagatttatactcaataaaatatatgaactatattgataaagattaataatgcagtgggtactgcacgattggggtgatgaacgatgtgtgaagctgttaaagaattgttggaactcattacctgtgggtggaaaagttttgataatcgagtttgttctcccgaatgaacttggtaacaatgctgaatcattcaatgcgttgattcccgatttactcctgatggctctgaatccaggcggtaaagagcgaacgatttccgaatacgatgatttaggcaaagcagctggattcataaaaactatacctatccctatctccaatggtcttcatgtcattgagtttcacaaatgaatggttattgagtgctttggtaattaaactaccaagataactacatccatttcatgcatttgctttttttttttcttttttttctttttttttctttttgttttgtattccaggtgtgaactagttagtgtgttgagtggacaaaagtaagtaatcgtattttgtgtt

SEQ ID NO: 18 - DNA, 1440 bp, Papaver somniferum
gaatcagaaactttcttctaaaatctttcaataccagtactgttagtttccgataagagccacactaatccattatggaaattcatttagaaagccaagaacaagaaatgaaatatcaatctcaaatctggaaccaaatatgtggcactgttgatacctctgttctgagatgtgcaattcaattaggtatatttgatgccattcataactctggcaaaccaatgattaccttaaccgaattatcaagcattgtttcatcaccctcttcatcttcaatcgaaccctgcaacttgtatagattagtgagatacttatcccaaatggatctcattagtatcggagaatgtttgaatgaagcaactgtttcattaacaggcacatccaagttactacttagaaaccaagaaaagagtttaattgattgggtattggcaatttcttgcgaaatgatggttgttgtttggcacgaactaagtagctctgtttcaactcctgcggatgagcctccaatcttccagaaggttcatggtaaaaatgctttagaattagcaggggaatttccagaatggaatgatctgatcaacaatgctatgactagtgatactagtgtaactaagccagcgctaatacaaggatgtggcaaaatcctgaacggagttacatcgttaattgatgtcggtggtggtcacggtgccactatggcctacatagttgaagcttttcctcacataaaaggtgcggtaatcgatttaccacatgttgttgaagccgctccggagcgtccaggtgttgagttcatcagcggtgatatattcaagtccatttctaacgctgatgctgtgttgttgaaggtatgtaaagagtagctaaccttagtgcgtctaatttattccacaaatttttctgatgcattttattcttatttttggtttttgcagtatgtcctgcacaattgggaagatacggaatgtgtgaatttactgaagagatgtaaggaagcagttccggcagacaaaggaaaagtgatcataatggatttagtaatagacgacgatgataacagtattttaacgcaggcaaagttgagccttgatctcactgtgatgaaccatggaggaggtagagaaaggactaaagaagattggagaaatctaattgagatgtctggatttagtaggcatgaaataattccaatatctgccatgccatcaattattgttgcttatccttagttaagtcacccgcatgtttacttgaacgggaataagttgggggcgtgttgaatctgttaacatcgcaattgtgcctttactttatgcattctcattccggtagaaactgtttggggcattcggattctgctgagcccttttatgtatgtttgtttgttggttggttggttttcaagtaactgaagtttcttctctgttttcaaggcat

SEQ ID NO: 19 - DNA, 1436 bp, Papaver somniferum
aagttgcaggtagggttatgagcaagctcaattatctctcctataaaagctaacattagaaaaactaataagcacacaaaccgtaaaagttctgaagatagacaaaacaagagaaaaaagatggaagtagtaagtaagattgatcaagaaaaccaagcaaaaatttggaaacaaatttttggttttgcagaatcattagttctaaaatgtgcagttcagttagagattgctgaaacacttcataataatgtaaaacccatgtctttatccgagttagcatctaaacttccggctcaacccgttaatgaagaccgtttgtaccgaattctgcatttcttagttcacatgaaactcttcaacaaagatgctaccacacagaaatattcattagctccaccagcaaagtatttgctaaaaggctgggaaaaatcaatggttccttcaatattaagcgtgactgataaagattttacagctccatggaatcatcttggggacggtttaaccggtaactgtaacgcttttgagaaagcgttaggaaagggcattcgggtttatatgagagaaaatcctgaaaaagatcaattgtttaatgaaggaatggcttgtgatactagattatttgcttcagcattggttaacgagtgcaaaagtattttcagtgacgggatcaatacacttgccggtgttggccgtggtactggtactgcagtgaaagccatatccaaagcttttccggatattaagtgcacaatccatgatcttcctgaagttaccagtaaaaatagtaaaattccaagagatgtttttaagtccgttcctagtgcagacgccatctttatgaaggtaacttctaagaaattttgttttagaatattcgttgcaactctaattgacaacattcataaaaaatatgttaatggtcttaatttattaattctagtagagttacttaaatgatatacaaaaattcaaaatcatataacatttgcagagcattcttcacgaatggaacgatgaggaatgtattcaaatcttgaaacgatgcaaagaagcaataccaaaagggggcaaagttatcattgcggatgtcgtaatagacatggactcgactcatccgtattcaaaatctagactcgcaatggatttggctatgatgctccacacgggtggaaaagagagaactgaagaagattggaaaaaacttattgatgctgcaggttttgctagctgtaaaattactaaactatctgctctccagtctgttattgaggcttaccctcattgaggataatttttatccttctgttttccctttggttaattgttgccttctctttggatcatggttgcgtttataataaatgcagcgtttctttcctggcggtaagtgcaagaaagaaaaagcttccagaaacttccttgagtatgcctgg

SEQ ID NO: 20 - DNA, 1921 bp, Papaver somniferum
cttgagtcatgccttgatatgctcatattttagtttgtcatattcactataactataaatttcaatacaatttctaaaactcatcatcattcaagagagatacaaataccttgatatccttttatcatcaatggagttattcataaagttaccatttatccaaccaattcctttcagtattattcttgttactacagtttcgattgttctattatacagtgtcttcttctgggttactgataagaaaaagaagaggaagaaagcaccaaatgctgcaggggcatggccgttaataggtcatctccgtctattgatgaacgacaaggaaccgttgtatagagcactagggagcatggctgataagtacggacctgcattcaacatccgattaggtaaccaagaagttcttgttgtgagtaactgggagatggtaaaacagtgttttggtaatcaaaatgataagctattttcgaatcgtcaaactacattagctgcaaaatacatgcttaatcaaacaacttctagcggattcgcaccatatggaccatattggagagagctacgaaagataatggtgcagcaattactctctaaacaatctttagaatcgtggaaacatctgaaaatcaaagagatggatgcttcatttagtaaacttaacgagttatgcaacaacaacggtactggaacagctaccctaattaggatggacgaatggtttgctgagttgacgttcaacgtgatcgcaagaaatgtctttggctaccaaagtggcggaaggtcgacagcgcttacgaacggtaatatgatcatactccctcaatctgtatcaatttaaggaaatcattttggtcttgttattaacttgaattttctattaggagatacggaatcaaagggcgagaggtacaagaaaacattggaagaagcacttcatcttatgtcaatttttgcagtttcagacatatttccaagtctagagtgggtagatcggttaagaggccttataaggaatatgaaacgctttggagatgagctaaattcaattgcagggtgtcttattgaagagcaccgccaaaagagattacaatccgtatctaaaagtgataaaggagttggtgatgaacaagacttcgttgatgttctcttatcggttgctgaaaaatcgcaacttcctggagatgaccctgatttggtcatcaagtctatgattctggttaggctattgataccaagtctattgcaattttggtttatgtgcttgttctaactttcgtttactgcatatggatgtgcaggaaatcgtatcaggtgggagtgagaccacatcgtcaaccttaacttgggccctctgtctgttactgaaccatccgcatgtgttaaagaaggcaaaagaggaattagatacgcacgtaggaaaagataggcatgtagaagagtcagatacccctaagctcgtgtacattaatgcaattatcaaagaatcaatgcgattgtatccaaacggggcaatgcttgatcggttggcgttagaagagtgcgaagttggtggatttcatgtaccggccgggggacgcttatttgtcaatgtttggaagattcagagagatccgagtgtttgggagaatcctctggagtttaaaccagagaggtggtttttgagtaatggtgaaaagatggatgtggattacaaaggtcacaatcatgaattcataccatttgggataggtcggaggatgtgcgctggtatgctttgggcatcggaggtgattcatttggtgctgccccgtcttattcatgggtttgatatgaaagcagcaagtgccaatgggaaagtagatatggcagaaatggcaggcatggtgatttgttttaagaagacacctcttgaagttatggtcaatcctcgagagtagatgtt

SEQ ID NO: 21 - DNA, 1688 bp, Papaver somniferum
catgaaattctttatgcaaagagtcaatctgactcaagctagctagaatatataccaatcataaaagaaatgatcatgagtaacttatggattcttacgctcatttctaccatattagcagtctttgctgctgtgttaatcattttcaggagaagaatatcagcatccacaacggaatggcctgttggcccaaaaacattaccaatcataggtaacttgcacattcttggaggcactgctctccatgtcgtcttacataaacttgctgaagtttacggcagtgtaatgacgatatggattggtagttggaaacctgttattattgtttccgactttgatcgagcctgggaagttcttgttaacaaatcgtcagattattcagctcgtgaaatgcctgagatcactaaaatcggcactgcaaattggagaacaatttcaagttctgattctggtccgttttgggccactcttcgaaaaggtcttcagagtgtagcattatcgcctcagcatttagcatcgcaaactgcacaccaagagagagatataataaagttgatcaaaaatttgaaagacgaagcagcttctggaatggttaaaccacttgatcatctcaagaaagcaactgtaagattaatcagtcggttaatctatggtcaggattttgatgacgataagtatgttgaagatatgcatgacgtgatcgagtttttgattcgtattagtggttatgctcaacttgctgaggtattctattatgctaaatatctaccaggtcataagagagctgtaactggcgccgaagaagcaaaaagaagagtaatagctctggtgcgtccttttcttcagtcaaaccctgctactaacacttacttgcattttctcaaatcgcaactgtatcctgaagaggttatcatattcgctatattcgaagcttatcttttaggtgttgatagcacttcttcaaccactgcatgggcactcgcattcttaatacgcgaaccatctgttcaagagaaactttatcaagagcttaagaatttcacagccaataacaatcgcacaatgctgaaagtcgaagacgtcaacaaattaccatatttacaagctgttgttaaagaaacaatgaggatgaaaccaattgcaccactggcgattcctcataaagcttgtaaagacacttcattgatgggcaagaaagttgataagggaactaaagttatggttaacattcatgctttacatcatactgaaaaggtttggaaagaaccttacaaattcataccagagaggtttctgcagaagcacgataaggcgatggaacaatcactattaccatttagtgcaggtatgagaatttgtgcaggaatggaattaggaaaacttcagtttagtttttctcttgctaatcttgttaatgcttttaaatggtcttgtgtgtctgatggagtgcttcctgatatgagtgatttactggggtttgttctgttcatgaaaaccccactcgaagcacgtatagttcctcgtttgtagtgatggaaatttcatctcatgttgttgtttctcttcatgtttactatttcgtactcgtttggttttggtgtaaaaaataagatctaaacttccaaatatcattaatgtttacacaaatcgaaatcaatcaactatgttatgaaaattagtgttttctc

SEQ ID NO: 22 - DNA, 2918 bp, Papaver somniferum
aagtgtgccactaatctactgctagtgctactgctcactgacacttacacatatgattgatttatggctaaacaggatgaccactaaatttattttggaaagcggagtgaattaattaagtggcacattttccatgagaattattgatggcatgcatttagatgaacaagatacaccaaatgtagtgactgaacaagatgctcgatcctaaccccacctgcaactttagctaaactttaataattacatgtcttatctttttattgaatcattttatctatcaatggatgctgatcaataatatcatatatctttgctttttcttcaatcatttagatgaacaaaaaacacaataagtgtagtggttgttcataaccccaccttcaactcattcttccctttaataacaaatatctttgctttttctccaatcatttacttgaacaaccaacactagtaagtgtagtggtttctcataaccccacctgcaatttttgcttacctttaataacatatatctttgattttcttcgatcattttagctaccaatggatgctgatccaaaaagttatggcaaaaagagacaacgtgatcgaacacgagcctctcgtgcaccacagcatcaaggtttgtggaaattaaccgcttgtaaaaaatggagtgcgtgatcataatgaggtattgctaagatatagtatcaactttagtgaactgggccaacaaaactcacgagttgttgaaaattggagattatatttataagataaaagggtcactccctacacaacgacttgcactgcaagtgaaaaagaaaaaaaacaaacaacctcaatctagctagagtcgtgaaaaagttttgtgcgactgttatttagttaattataaaatttcaatgaagtcgttaatgatgaacaagttattatttctccaacggattactgattctccttcgaccaccattatcagtacttttattgttacaataatatccattgtttttctctacactgtcttgttgataaggacgactaagaataagcagaagatagcagcaccaaaagcatcgggggcgtggccgttcataggtcatctcaaactattcatgaaacaagatactcagttttacagaactctaggaaccatgtctgataaatacgggtcggtgttcacacttcgattaggaaaccaagcaatcctagttgtgagcaactgggagatggtaaaagaatgtttcacaacaaacgacaagtcattctcgaatcgtccaagtacgttaagcactaaatacatgctgaatgacactaattctgtcgtgttttcaccttacggaacgtattggagagaaatgcggaagatattggtgcaaaaactactgatctctaaccaaagatcagaggcattgaaaaatctgaaaacgaaagaaatcgacaactcgtttgtaaagcttaatgatttatgcaacaacgatgtcagtggaggaggcacaaaagttaggatggacgaatggttggctgacatgatgttcaacattattgctaggattacatttggttaccaaagcggaggaggcgatgcacctggtatgtgatcatcaaattttcgttaaaaccaaattaacttgtactatatcttatgtttacatgttatattgatcactttgacacgttctgatcattttcacaaatcgaattaggcgcttctacaacatccaagaatgtcgagagatacaagaaaacgttggacgagatgtttgttgttttagcgacgaggtttgcagtttcagatatatttccatctctggagtttatagaccgattgagaggtcttgtaaaggatatgaaaatcttgggagacgaattaaactccattgctggatgttttattgaagaacatcgtcaaaagagacgagaatcattatcctcattgttatctttgtcaaatgaatccgttggtgatgaacaagatttcattgatgttctcttgtcaataatggatcagtcacggcttcccggagatgacccagattttattatcaaaattatgatcctggtaacatatattacaacagtatttctttaagttatggattaatggatgtcgtaaccatgaatatttttctgatctggataaatgtaatccggaactaatatatgaatattgttgacgcaggaagcttttgcaggtgggacggacagtttaagtgcaaccttaacttgggtcctctctctactgctgaaccacccaaacgtgttaaagagggcaagggaggaaatagataggcatgtggaaaacggtaagcaagtggaagtgtctgatattccgaagctcggatacattgatgcaataatcaaagagacgatgagattgtatccagtcggagcattaagcgaacgatacacgactgaagaatgcgaggttggtcggtttaacgtacccgctggcacacgcttactggtgaatatatggaagatccacagagacccaagtgtgtgggagaatccatcagattttcaaccagagaggtttttgtgcagcgataaggtgggtgtggatttatatggccagaattatgagctgataccatttggggccggtaggagggtatgtccggctatagtttcatcactgcagacgatgcattatgcgttggcgcgtcttattcaaggatatgaaatgaaatcagccagcctcgatgggaaggtgaatatggaagaaatgatagccatgtcgtgccacaagatgagccctcttgaagttattatcagtcctcgggagccgaggcggagttaaatcttatgttccaattttacattagcatctttgattatgaaatgtattgctcttaagtttcttttttgttttttatatttttaagcttgtatgtgatcatcagcgaaaatgatgatgacagaatcgt

SEQ ID NO: 23 - DNA, 1915 bp, Papaver somniferum
ttcagttcattcatggcgtatttgatgatcaagaagtctatctatttgttttttgatcaaccaactgcagttggcactcttatacttgcttttctgctgacactttcgcctgttattatttactatgaacagaagaagaggggtttgaggcgaaatcgcaccgcaattacaacgactccattaccagaggcatcaggtgcatggccagtgataggtcatcttcttcttttcatgaacgaaaacgatctaaatcatgtaactcttggtcacatggctgataaatatggacctattttcagcttaagattcggtagacatagaactctagttgttagtagttgggagatggtaaaggagtgttttacaggtaccaatgacaagttgttctcaaatcgtccttcctccttggcggttaaacttatgttttatgacactgaatcttatggttttgcaccttatgggaaatactggagagagttgcgaaagatatctacacacaaactcctctctaatcagcaattagagaagttcaagcacttgcggatttctgaagtcgataactcctttaaaaagcttcatgagttatgcagcaacaacaaacagggaggtgatactacatatgtggctagtcttgtgagaatggatgattggttcgcgtacttgacatttaacgtaataggacggatcgtcagcggattccaatcaaatgcagtggcaggtgagctcatatagctaggtttttatatgtttggtttgtacacacacagctcattcatattctaaactgaattatatgttataattgaacaacataggtgccacaaacagccaggaaaaatacaagcttgcaatcgatgaagtgtcaaatcttatggcaacgtttgccgtttcagatgtggttccacggcttgggtggattgatcgattgactggtcttacaggaaagatgaagaattgtggtaaaaaattagatgcagtagttggggatgcagtggaggatcatcgccaaaagaaactcaaaatttctagaaataacacaggagcacttacggagcacgaagaagaagactttatcgatgtttgcttgtcgattatggagcagtcacagattccgggaaaccaccccgaaatctctgtcaaatctattgccttggtaatacgtctcataagcatgttagcagattttacctctatatatacttacatattattttttatcaatcacacatatgtgcaggacatgttatcgggtgggagtgacactacaaaattgataatgacatggaccctttctttgctgttgaaccatccagacatattggacaaggctaaagaagaagtagatacatacttcgggaagaaaaagatatcggataacacacctgtggttgatgctgccgatgttcctaacctcgtctacatccaagcaatcatcaaagaatcaatgcggttataccctgctagcacattgatggagcgaatgacaagtgatgattgtgatgttggtggcttccacgtaccagctgggacacgattatgggttaacgtatggaagatgcaacgggacccaagggtgtggaaagatccactggtatttctacctgagagattcttgagcaatgacaaagggatggtagatgtgaagggtcagaattatgaactgataccatttggaacaggcaggcggatatgtcctggtgcatcttttgccttggaagtcttgcatttggttcttactcgtcttattcttgagttcgagatgaaggcaccagaggggaaaattgacatgagggcaagaccaggttttttccacaacaaggtggtgccactagatgttcaactcaccccacgcacactagattaagattcctatatatgctaattaattagatgaataaaatctgtggtcgagtaa

SEQ ID NO: 24 - DNA, 1572 bp, Papaver somniferum
cgcatataatccaatttgcattgtttatcgaccttgaggaacaattaggggatatggcaacaatgtctagtgctgctgtagaagtgatctcgaaagaaacgattaaaccaagaaatccaacaccatatcaacttagaaactacaatatgtcacttctcgaccaatattcttctctagtttatgttccgatcattcttttctaccctgctgcctccgacgctaatagtaccggaagtaagcaccatgatgatcttcacttgcttaagaggtctctttctgaaacgctagttcacttttatccaatggctggtaggatgaaagacaacatgactgttgactgtaacgacgaaggtattgactttttcgaagtaagaatcaaaggtagaatgtgtgacttcatgatgaaatcagatgcacacttaagtctgcttcttccgtctgaagtcgcttccacgaacttcgtgaaggaagcacaggtgattgttcaagtgaacatgtttgattgcggtggaactgccatttgtttctgtatatcaaacaagattgcagatgcatgcaccatgattaccttcattcgtagtttggcaggcaccaccaacatagctcgtcgtgggagctctattgctgcaccaaccacaaatcagaatttggttccttctttcgattcgacatcactctttccacctagtgaacaattggcatctcaagtttcctatcctacacaggatagtaccagcgtagataaacttgtcagcaaaagatttgtgtttgatgcggcaaagattacatctgcacgtgaaaaattgcaatccttgatgcatgataaatacaaatgccataggccgacaagggttgaggtagtttccgctttgatatggaagtcagcagtgaaatctgctccgcccggttctatatccactgtaacccatgccatgaactttagaaagaaaatggatccaccattacaagatgcgtcattcgggaatctttgtgtggttgttacagcagtattaccagcaacaacggcgacaacaacaaatccagcaaccaaaaaagttagtagtacgagtaatgaagagcaagtggcacttgatgagttaagtgattttgtagccctattgaggcgcgaaatagataaggtaaagggtgataaaggttgcatggagaaaatcattcaaaagttcatctatggtcatgatgcttccgtagcgaaagacagtgatgttgaagataaggtgacagctttgtttatgactagctggtgcaagtttggattctacgaagctgattttggttggggaacgccagtttgggtaactactgttccattaattgagccaaagtacaagaacatggttttcatgaacgatatgaaatgtggtgaaggaattgaagtgtgggtgaattttctggaggatgatatgaccaagttcgaacaccacctaagagagatcctccaactgttttgattttcaaccgtttccctaatagaggtcaattgtcgtgtttgtccatcttaactaccatctttattctcttgttttcatacttgtatttgtcttactccggtaa

SEQ ID NO: 25 - DNA, 2488 bp, Papaver somniferum
ctaacaggcaaacaataacaggttgcacctacaacattcaatttttattttggtaaatgaagttcagttggagagtaaccacatctttgttgtcggcattgcccccacaatactgagtgttttggctgagtgtagtctgactgtaggtaagctacaactgcatgttgcagataataatcactaactgattattcatgcatacctaacagtcatattgttatagttcccaaaaaaaattctcgaactataaaggcatgcatggacagaaaaatatatcagagagatatcagaaattcaaagagatggaaggaacagggaagatagtatgtgtaacaggtggagctggatacttggcatcttggctgatcatgagattgcttgaacgtggttactctgttcggaccaccgttcggtctgacccaagtacgtaataaattaaatttcctggcatcattttcttcaatataaatttcttattatctagttcatcattctttattgttccaatcatgtccccccaagtctaaaagaagtagtaatctaaaaatagctaatttatgtacgaaattgtaacaatgatctcctagcttatgaggctcacctaatttcgtttctatcattttgtgtcttgaaagaatttagggaagatgtgagccaccttaaagctcttcctgaagctacagagaagcttcaaatttttgaagcagatcttgaaaacccagaaagtttcgacgatgcgatcaacggttgtgtcggtgtctttctcgttgctcaaggaatgaattttgccgaagaatatactcttgaaaaaataatcaaaacatgcgtggaaggaactcttagaattctacagtcatgcttgaaatctaaaacagtgaaaaaggttgtgtacacatcttctgctgatgcagcaatgatgataagtaatctcaaagctgttaaagaaattgacgagacaatatggtcagaagttgacaatttcattagcaaaccggaacaagttattcctggattgccctcatatgtggtttcaaaggtactgacagaaagagcttgcctaaagttttctgaagaacatggtttggatgttgttactatacttcctccgttggttgttggaccttttatcactccccatcctcctcccagtgtatctatagctctttcgataatttcaggtatcctctccatccgaaaaatatgccaattcctaaacttaaaaggcatattgatatttaataatacctccatacctaaaaaaagagttgctatataacatttttaattttcgcccatttttaggcctaattgaaaaagttataataacattttaggaaggagggagaatgatttttgagcaaaccttagaactgtgtggtgagatttgtccgttatcattgttggtataactgtgtatatcatggtttttaaaagcgccgctcacgctacgcttcgtacggttcggtctagatttttttaattcgctccgaagcgtagttatgaagctaccatgaagcgccgcttcacgctacgtttcgtacgcttcgcttcagatttttcaaattcgctccgaggcgaatctaccatgaagtggaagattcctttaattgattcacttttttacttagtcaagtcttttttagggggtttcgaaaactaaagtgaaccactgcgcctcgctactgtttttgaaattaactagacttatattaaattgatacaattattatatcttcctaaatattaaattattaataacaaactactactatttataggaaaaaattcgcttcaaatatcaatcataaaacgacgcttcacatttcaacatgcgcatcgcttcgtataaaaaaaaaacgcttcacgctttcaataccttggtgtacatagattaatacttcctcctctgcgctggtgttaacatttctgtgtttcgtttatatatatgaccaggtgatgtgtcgatgatgcttggtgttagacttgaaaatgcggtacatatagatgatgttgctttagcacacatattcgtttttgaatgtgaaaaagcaaaaggaagacatatttgttcttcagttgattttccaatgcatgatctgcctaaatttatatctgagaattatccggaattcaacgtaccgactgagtgagtttatctttcaccaccttctttattattattcatcaagtcactttgggtattttaaccttattgtttttactgaattatcatcagtttactaaaggatattgaggaacaagaaccagttcatctttcctcagataagctgttgagtatgggatttcagttcaaatatgattttgcagagattttcggtgatgcaatacgatgtgccaaagagaagggtttcctttagagaccaactatagtttggttcggaggagatgtgggagtagctagcccaaaatgccctgctcgcactagcttatattattgttattgtttttcaaatgaataaacgggcag

SEQ ID NO: 26 - DNA, 1133 bp, Papaver somniferum
aataaaaatccaacaatggcagatccttatgaattcctaatgtgcattcacaatcctgaagaagataccctaacaagaaattttccgattcctgctactcccttagatcaaaacaccaaagacatttctttaaatcctgataggaaaacctcacttcgaatctttcggccaccaaccaaagaacctcctgtaacaaagaataagctgcttcctatcataatttatttccatggtggaggtttcattcttttcaatgcagattcaactatgaaccatgacttttgtcaatcgattgctacacatatacccgcgctggtcgtttctgtagactaccgtcttgctcctgaaaaccgacttcccgctgcctatgatgatgctgttgatgctttaaactgggtcaaagaccaaggtttaggcaaactaaataatagtgaagtatggttaaaagagtatggtgacttctcaaagtgtttcattatggggtgcagctcaggtgctaatgttgcatatcatgccagtttaagagcaatagaaatggatcttgaaccagctaagattaatggattaatattacactgccctttttttggtagtcttgagagaactgaatcagattcaaaagtgatcaacaatcaggacttgccgcttgccgtaagggatgtcatgtgggaactggcgttgccgcttgggtctactcgtgatcacgtttattgtaatccgaatattgatcatgatggatcatcatctggaaatatggtggggttaatcgagagatgttttgtggtaggattttatggggatccacttattgatcgacaaattcagctggtgaagatgctggaggaaaaaggtgtgaaggttgaaacttggattgaacaaggagggtatcatggggtgctatgctttgaccctatgatacgtgaaacctttttggaaaaactaaaacattttattttaaacgacgaatttatatactaaaatatattattagtattaaacaatgaaattcttattttttctaaaatgagcttttggacgaaacattgtgtacgaactagctgatgtaatttttcgttttaccggatttttcattttttttgctttctttctgctctcttttataagtcgttctt

SEQ ID NO: 27 - protein, 900 aa, Papaver somniferum
MELQYISYFQPTSSVVALLLALVSILSSVVVLRKTFLNNYSSSPASSTKTAVLSHQRQQSCALPISGLLHIFMNKNGLIHVTLGNMADKYGPIFSFPTGSHRTLVVSSWEMVKECFTGNNDTAFSNRPIPLAFKTIFYACGGIDSYGLSSVPYGKYWRELRKVCVHNLLSNQQLLKFRHLIISQVDTSFNKLYELCKNSEDNQGNYTTTTTAAGMVRIDDWLAELSFNVIGRIVCGFQSGPKTGAPSRVEQFKEAINEASYFMSTSPVSDNVPMLGWIDQLTGLTRNMKHCGKKLDLVVESIINDHRQKRRFSRTKGGDEKDDEQDDFIDICLSIMEQPQLPGNNNPSQIPIKSIVLDMIGGGTDTTKLTTIWTLSLLLNNPHVLDKAKQEVDAHFRTKRRSTNDAAAAVVDFDDIRNLVYIQAIIKESMWLYPASPVVERLSGEDCVVGGFHVPAGTRLWANVWKMQRDPKVWDDPLVFRPDRFLSDEQKMVDVRGQNYELLPFGAGRRVCPGVSFSLDLMQLVLTRLILEFEMKSPSGKVDMTATPGLMSYKVIPLDILLTHRRIKPCVQSAASERDMESSGVPVITLGSGKVMPVLGMGTFEKVGKGSERERLAILKAIEVGYRYFDTAAAYETEEVLGEAIAEALQLGLVKSRDELFISSMLWCTDAHADRVLLALQNSLRNLKLEYVDLYMLPFPASLKPGKITMDIPEEDICRMDYRSVWAAMEECQNLGFTKSIGVSNFSCKKLQELMATANIPPAVNQVEMSPAFQQKKLREYCNANNILVSAISVLGSNGTPWGSNAVLGSEVLKKIAMAKGKSVAQVSMRWVYEQGASLVVKSFSEERLRENLNIFDWELTKEDHEKIGEIPQCRILSAYFLVSPNGPFKSQEELWDDEA

SEQ ID NO: 28 - protein, 901 aa, Papaver somniferum
MELQYISYFQPTSSVVALLLALVSILSSVVVLRKTFLNNYSSSPASSTKTAVLSHQRQQSCALPISGLLHIFMNKNGLIHVTLGNMADKYGPIFSFPTGSHRTLVVSSWEMVKECFTGNNDTAFSNRPIPLAFKTIFYACGGIDSYGLSSVPYGKYWRELRKVCVHNLLSNQQLLKFRHLIISQVDTSFNKLYELCKNSEDNHGNYTTTTTTAAGMVRIDDWLAELSFNVIGRIVCGFQSGPKTGAPSRVEQFKEAINEASYFMSTSPVSDNVPMLGWIDQLTGLTRNMKHCGKKLDLVVESIINDHRQKRRFSRTKGGDEKDDEQDDFIDICLSIMEQPQLPGNNNPSQIPIKSIVLDMIGGGTDTTKLTTIWTLSLLLNNPHVLDKAKQEVDAHFRTKRRSTNDAAAAVVDFDDIRNLVYIQAIIKESMWLYPASPVVERLSGEDCVVGGFHVPAGTRLWANVWKMQRDPKVWDDPLVFRPDRFLSDEQKMVDVRGQNYELLPFGAGRRVCPGVSFSLDLMQLVLTRLILEFEMKSPSGKVDMTATPGLMSYKVIPLDILLTHRRIKPCVQSAASERDMESSGVPVITLGSGKVMPVLGMGTFEKVGKGSERERLAILKAIEVGYRYFDTAAAYETEEVLGEAIAEALQLGLVKSRDELFISSMLWCTDAHADRVLLALQNSLRNLKLEYVDLYMLPFPASLKPGKITMDIPEEDICRMDYRSVWAAMEECQNLGFTKSIGVSNFSCKKLQELMATANIPPAVNQVEMSPAFQQKKLREYCNANNILVSAISVLGSNGTPWGSNAVLGSEVLKKIAMAKGKSVAQVSMRWVYEQGASLVVKSFSEERLRENLNIFDWELTKEDHEKIGEIPQCRILSAYFLVSPNGPFKSQEELWDDEA

SEQ ID NO: 29 - protein, 900 aa, Papaver somniferum
MELQYISYFQPTSSVVALLLALVSILSSVVVLRKTFLNNYSSSPASSTKTAVLSHQRQQSCALPISGLLHIFMNKNGLIHVTLGNMADKYGPIFSFPTGSHRTLVVSSWEMVKECFTGNNDTAFSNRPIPLAFKTIFYACGGIDSYGLSSVPYGKYWRELRKVCVHNLLSNQQLLKFRHLIISQVDTSFNKLYELCKNSEDNQGNYPTTTTAAGMVRIDDWLAELSFNVIGRIVCGFQSGPKTGAPSRVEQFKEAINEASYFMSTSPVSDNVPMLGWIDQLTGLTRNMKHCGKKLDLVVESIINDHRQKRRFSRTKGGDEKDDEQDDFIDICLSIMEQPQLPGNNNPSQIPIKSIVLDMIGGGTDTTKLTTIWTLSLLLNNPHVLDKAKQEVDAHFRTKRRSTNDAAAAVVDFDDIRNLVYIQAIIKESMWLYPASPVVERLSGEDCVVGGFHVPAGTRLWANVWKMQRDPKVWDDPLVFRPDRFLSDEQKMVDVRGQNYELLPFGAGRRVCPGVSFSLDLMQLVLTRLILEFEMKSPSGKVDMTATPGLMSYKVIPLDILLTHRRIKPCVQSAASERDMESSGVPVITLGSGKVMPVLGMGTFEKVGKGSERERLAILKAIEVGYRYFDTAAAYETEEVLGEAIAEALQLGLVKSRDELFISSMLWCTDAHADRVLLALQNSLRNLKLEYVDLYMLPFPASLKPGKITMDIPEEDICRMDYRSVWAAMEECQNLGFTKSIGVSNFSCKKLQELMATANIPPAVNQVEMSPAFQQKKLREYCNANNILVSAISVLGSNGTPWGSNAVLGSEVLKKIAMAKGKSVAQVSMRWVYEQGASLVVKSFSEERLRENLNIFDWELTKEDHEKIGEIPQCRILSAYFLVSPNGPFKSQEELWDDEA

SEQ ID NO: 30 - DNA, 2703 bp, Papaver somniferum
atggagctccaatatatttcttattttcaaccaacttcctccgttgttgctcttctacttgctcttgtatccatcttatccagtgtcgttgttttgaggaagacatttttgaataactactcatcatcacctgcatcatccacaaaaacagcggtactttctcatcagcggcagcagtcgtgtgcattgccaatttccggtctcctccatattttcatgaataaaaacggcttaattcatgtaactcttggaaatatggctgataaatacggtccgattttcagtttcccaacaggtagccatagaactctcgttgtgagcagttgggagatggtaaaagagtgttttactggcaacaatgacactgctttctcaaaccgtcctatcccgttagcttttaagactatattttatgcatgcggtggcatagactcatacggtctttcgagtgtaccttatggaaaatattggagggagcttcgaaaggtctgtgtgcataacctcctgtctaatcaacaactactcaagttcagacacttgataatttctcaagtcgatacgtctttcaataagctgtatgagttatgcaaaaactctgaagacaaccagggaaactatactactactactaccgcagctggcatggtgagaatcgatgattggctcgccgaattatcgttcaatgtgataggaagaatagtctgcggattccaatcaggccctaagacaggtgctccaagcagggtggaacaatttaaagaagcaattaatgaagcatcttattttatgtcgacatctccagtgtcagataatgttccaatgctagggtggattgaccaattgacaggtcttacgagaaatatgaagcactgcggaaagaaattagacttggtggtcgagagcataattaatgatcatcgtcaaaagagacgattctctagaactaaaggaggagatgagaaggacgatgaacaagatgacttcatcgacatttgtttgtcaataatggagcaaccacagcttcctggcaacaataatccttctcagatacctatcaaatctattgtcctggacatgataggtgggggcactgacaccacaaaactgaccaccatctggaccctttccttgctgctgaacaacccccatgtgttggacaaggcaaaacaagaagtggatgcacactttcgaaccaaaaggagatcaacaaatgatgcagcagcagccgtggtggattttgatgatattcgtaaccttgtctacatccaggcaatcatcaaagaatcaatgtggttgtatccagccagccccgtggtggagcgactgagcggcgaagattgtgtggtcggtgggtttcatgtaccagcagggacgagattatgggctaacgtatggaagatgcaacgagaccctaaagtatgggatgatccattggtgtttcgaccagacagatttttgagcgatgaacagaagatggttgatgtaaggggtcaaaattatgagctgttaccatttggagccggtcgacgtgtatgtccaggtgtatccttctctttggatctaatgcaactggtactgactcgtcttattctcgagtttgaaatgaagtctcctagcgggaaagtggacatgacagcaacaccaggattaatgagttacaaggtgatcccccttgacattctgctcacccatcgtcgcataaagccgtgtgtgcagtcagcagcctctgagagagacatggagagtagtggtgtaccagtaatcactctgggctcgggcaaggtgatgcctgttctgggcatgggaacatttgagaaagttggtaaagggtccgaaagagagaggttggcgattttaaaagcgatagaggtgggttacagatacttcgatacagctgctgcatacgaaactgaagaggttcttggagaagctattgctgaagcacttcaacttggcctagtcaaatctcgagatgaacttttcatcagttccatgctctggtgcactgatgctcacgctgatcgtgtcctcctcgctcttcagaattcgctgaggaatcttaaattggagtatgtggatctatatatgttacccttcccggcaagcttgaagcctgggaagataacgatggacataccagaggaagatatttgtcgcatggactacaggtctgtatgggcagccatggaagagtgtcaaaaccttggcttcactaaatcaatcggtgttagcaatttctcctgcaaaaagcttcaggaattgatggcgaccgccaacatccctccagctgtgaatcaagtggagatgagcccggctttccaacaaaagaagctgagagagtattgcaacgcaaataatatattagtcagtgcaatctctgtactgggatcaaacggaaccccatggggctccaatgcagttttgggttctgaggtgcttaagaaaattgctatggccaaaggaaaatctgttgctcaggttagtatgagatgggtttacgagcaaggcgcgagtcttgtggtaaaaagtttcagtgaagagagattgagggaaaacttgaacatatttgactgggaactcactaaggaagaccatgaaaagatcggtgagattccacagtgcagaatcttgagtgcttattttttggtctcacctaatggacctttcaaatctcaagaagagttgtgggatgatgaagcttga

SEQ ID NO: 31 - DNA, 2706 bp, Papaver somniferum
atggagctccaatatatttcttattttcaaccaacttcctccgttgttgctcttctacttgctcttgtatccatcttatccagtgtcgttgttttgaggaagacatttttgaataactactcatcatcacctgcatcatccacaaaaacagcggtactttctcatcagcggcagcagtcgtgtgcattgccaatttccggtctcctccatattttcatgaataaaaacggcttaattcatgtaactcttggaaatatggctgataaatacggtccgattttcagtttcccaacaggtagccatagaactctcgttgtgagcagttgggagatggtaaaagagtgttttactggcaacaatgacactgctttctcaaaccgtcctatcccgttagcttttaagactatattctatgcatgcggtggcatagactcatacggtctttcgagtgtaccttatggaaaatattggagggagcttcgaaaggtctgtgtgcataacctcctgtctaatcaacaactactcaagttcagacacttgataatttctcaagtcgatacgtctttcaataagctgtatgagttatgcaaaaactctgaagacaaccatggaaactatactactactactactaccgcagctggcatggtgagaatcgatgattggctcgccgaattatcgttcaatgtgataggaagaatagtctgcggattccaatcaggccctaagacaggtgctccaagcagggtggaacaatttaaagaagcaattaatgaagcatcttattttatgtcgacatctccagtgtcagataatgttccaatgctagggtggattgaccaattgacaggtcttacgagaaatatgaagcactgcggaaagaaattagacttggtggtcgagagcataattaatgatcatcgtcaaaagagacgattctctagaactaaaggaggagatgagaaggacgatgaacaagatgacttcatcgacatttgtttgtcaataatggagcaaccacagcttcctggcaacaataatccttctcagatacctatcaaatctattgtcctggacatgataggtgggggcactgacaccacaaaactgaccaccatctggaccctttccttgctgctgaacaacccccatgtgttggacaaggcaaaacaagaagtggatgcacactttcgaaccaaaaggagatcaacaaatgatgcagcagcagccgtggtggattttgatgatattcgtaaccttgtctacatccaggcaatcatcaaagaatcaatgtggttgtatccagccagccccgtggtggagcgactgagcggcgaagattgtgtggtcggtgggtttcatgtaccagcagggacgagattatgggctaacgtatggaagatgcaacgagaccctaaagtatgggatgatccattggtgtttcgaccagacagatttttgagcgatgaacagaagatggttgatgtaaggggtcaaaattatgagctgttaccatttggagccggtcgacgtgtatgtccaggtgtatccttctctttggatctaatgcaactggtactgactcgtcttattctcgagtttgaaatgaagtctcctagcgggaaagtggacatgacagcaacaccaggattaatgagttacaaggtgatcccccttgacattctgctcacccatcgtcgcataaagccgtgtgtgcagtcagcagcctctgagagagacatggagagtagtggtgtaccagtaatcactctgggctcgggcaaggtgatgcctgttcttggcatgggaacatttgagaaagttggtaaagggtccgaaagagagaggttggcgattttaaaagcgatagaggtgggttacagatacttcgatacagctgctgcatacgaaactgaagaggttcttggagaagctattgctgaagcacttcaacttggcctagtcaaatctcgagatgaacttttcatcagttccatgctctggtgcactgatgctcacgctgatcgtgtcctcctcgctcttcagaattcgctgaggaatcttaaattggagtatgtggatctatatatgttacccttcccggcaagcttgaagcctgggaagataacgatggacataccagaggaagatatttgtcgcatggactacaggtctgtatgggcagccatggaagagtgtcaaaaccttggcttcactaaatcaatcggtgttagcaatttctcctgcaaaaagcttcaggaattgatggcgactgccaacatccctccagctgtgaatcaagtggagatgagcccggctttccaacaaaagaagctgagagagtattgcaacgcaaataatatattagtcagtgcaatctctgtactgggatcaaacggaaccccatggggctccaatgcagttttgggttctgaggtgcttaagaaaattgctatggccaaaggaaaatctgttgctcaggttagtatgagatgggtttacgagcaaggcgcgagtcttgtggtaaaaagtttcagtgaagagagattgagggaaaacttgaacatatttgactgggaactcactaaggaagaccatgaaaagatcggtgagattccacagtgcagaatcttgagtgcttattttttggtctcacctaatggacctttcaaatctcaagaagagttgtgggatgatgaagcttga

SEQ ID NO: 32 - DNA, 2703 bp, Papaver somniferum
atggagctccaatatatttcttattttcaaccaacttcctccgttgttgctcttctacttgctcttgtatccatcttatccagtgtcgttgttttgaggaagacatttttgaataactactcatcatcacctgcatcatccacaaaaacagcggtactttctcatcagcggcagcagtcgtgtgcattgccaatttccggtctcctccatattttcatgaataaaaacggcttaattcatgtaactcttggaaatatggctgataaatacggtccgattttcagtttcccaacaggtagccatagaactctcgttgtgagcagttgggagatggtaaaagagtgttttactggcaacaatgacactgctttctcaaaccgtcctatcccgttagcttttaagactatattctatgcatgcggtggcatagactcatacggtctttcgagtgtaccttatggaaaatattggagggagcttcgaaaggtctgtgtgcataacctcctgtctaatcaacaactactcaagttcagacacttgataatttctcaagtcgatacgtctttcaataagctgtatgagttatgcaaaaactctgaagacaaccagggaaactatcctactactactaccgcagctggcatggtgagaatcgatgattggctcgccgaattatcgttcaatgtgataggaagaatagtctgcggattccaatcaggccctaagacaggtgctccaagcagggtggaacaatttaaagaagcaattaatgaagcatcttattttatgtcgacatctccagtgtcagataatgttccaatgctagggtggattgaccaattgacaggtcttacgagaaatatgaagcactgcggaaagaaattagacttggtggtcgagagcataattaatgatcatcgtcaaaagagacgattctctagaactaaaggaggagatgagaaggacgatgaacaagatgacttcatcgacatttgtttgtcaataatggagcaaccacagcttcctggcaacaataatccttctcagatacctatcaaatctattgtcctggacatgataggtgggggcactgacaccacaaaactgaccaccatctggaccctttccttgctgctgaacaacccccatgtgttggacaaggcaaaacaagaagtggatgcacactttcgaaccaaaaggagatcaacaaatgatgcagcagcagccgtggtggattttgatgatattcgtaaccttgtctacatccaggcaatcatcaaagaatcaatgtggttgtatccagccagccccgtggtggagcgactgagcggcgaagattgtgtggtcggtgggtttcatgtaccagcagggacgagattatgggctaacgtatggaagatgcaacgagaccctaaagtatgggatgatccattggtgtttcgaccagacagatttttgagcgatgaacagaagatggttgatgtaaggggtcaaaattatgagctgttaccatttggagccggtcgacgtgtatgtccaggtgtatccttctctttggatctaatgcaactggtactgactcgtcttattctcgagtttgaaatgaagtctcctagcgggaaagtggacatgacagcaacaccaggattaatgagttacaaggtgatcccccttgacattctgctcacccatcgtcgcataaagccgtgtgtgcagtcagcagcctctgagagagacatggagagtagtggtgtaccagtaatcactctgggctcgggcaaggtgatgcctgttctgggcatgggaacatttgagaaagttggtaaagggtccgaaagagagaggttggcgattttaaaagcgatagaggtgggttacagatacttcgatacagctgctgcatacgaaactgaagaggttcttggagaagctattgctgaagcacttcaacttggcctagtcaaatctcgagatgaacttttcatcagttccatgctctggtgcactgatgctcacgctgatcgtgtcctcctcgctcttcagaattcgctgaggaatcttaaattggagtatgtggatctatatatgttacccttcccggcaagcttgaagcctgggaagataacgatggacataccagaggaagatatttgtcgcatggactacaggtctgtatgggcagccatggaagagtgtcaaaaccttggcttcactaaatcaatcggtgttagcaatttctcctgcaaaaagcttcaggaattgatggcgaccgccaacatccctccagctgtgaatcaagtggagatgagcccggctttccaacaaaagaagctgagagagtattgcaacgcaaataatatattagtcagtgcaatctctgtactgggatcaaacggaaccccatggggctccaatgcagttttgggttctgaggtgcttaagaaaattgctatggccaaaggaaaatctgttgctcaggttagtatgagatgggtttacgagcaaggcgcgagtcttgtggtaaaaagtttcagtgaagagagattgagggaaaacttgaacatatttgactgggaactcactaaggaagaccatgaaaagatcggtgagattccacagtgcagaatcttgagtgcttattttttggtctcacctaatggacctttcaaatctcaagaagagttgtgggatgatgaagcttga

SEQ ID NO: 33 - DNA, 966 bp, Papaver somniferum
atggagagtagtggtgtaccagtaatcactctgggctcgggcaaggtgatgcctgttctgggcatgggaacatttgagaaagttggtaaagggtccgaaagagagaggttggcgattttaaaagcgatagaggtgggttacagatacttcgatacagctgctgcatacgaaactgaagaggttcttggagaagctattgctgaagcacttcaacttggcctagtcaaatctcgagatgaacttttcatcagttccatgctctggtgcactgatgctcacgctgatcgtgtcctcctcgctcttcagaattcgctgaggaatcttaaattggagtatgtggatctatatatgttacccttcccggcaagcttgaagcctgggaagataacgatggacataccagaggaagatatttgtcgcatggactacaggtctgtatgggcagccatggaagagtgtcaaaaccttggcttcactaaatcaatcggtgttagcaatttctcctgcaaaaagcttcaggaattgatggcgaccgccaacatccctccagctgtgaatcaagtggagatgagcccggctttccaacaaaagaagctgagagagtattgcaacgcaaataatatattagtcagtgcaatctctgtactgggatcaaacggaaccccatggggctccaatgcagttttgggttctgaggtgcttaagaaaattgctatggccaaaggaaaatctgttgctcaggttagtatgagatgggtttacgagcaaggcgcgagtcttgtggtaaaaagtttcagtgaagagagattgagggaaaacttgaacatatttgactgggaactcactaaggaagaccatgaaaagatcggtgagattccacagtgcagaatcttgagtgcttattttttggtctcacctaatggacctttcaaatctcaagaagagttgtgggatgatgaagcttga

SEQ ID NO: 34 - DNA, 26 bp, artificial sequence
  primer wild type allele
ccaggcaatcatcaaagaatcaatgc

SEQ ID NO: 35 - DNA, 26 bp, artificial sequence
  primer mutant sequence
ccaggcaatcatcaaagaatcaatgt

SEQ ID NO: 36 - DNA, 21 bp, artificial sequence
  primer common primer
cacggggctggctggatacaa

SEQ ID NO: 37 - DNA, 23 bp, artificial sequence
  primer
cgactcactatagggagagcggc

SEQ ID NO: 38 - DNA, 24 bp, artificial sequence
  primer
aagaacatcgattttccatggcag

SEQ ID NO: 39 - DNA, 20 bp, artificial sequence
  primer
gcagtgcttcatatttctcg

SEQ ID NO: 40 - DNA, 25 bp, artificial sequnece
  primer
ccttatggaaaatattggagggagc

SEQ ID NO: 41 - DNA, 19 bp, artificial sequence
  primer
gtctctctcagaggctgct

SEQ ID NO: 42 - DNA, 20 bp, artificial sequence
  primer
ttgtctacatccaggcaatc